European Patent Application EP 4 137 567 A1, published February 22, 2023. Title: COELENTERAZINE-UTILIZING LUCIFERASES WITH STABLE GLOW-TYPE LIGHT EMISSION, INCREASED SUBSTRATE AFFINITY,SUPPRESED PRODUCT INHIBITION, AND MODULATED EMISSION WAVELENGTHS, AND METHODS OF PRODUCING AND USING THEREOF. Applicant: Masarykova Univerzita. The sequence listing filed with the application follows.

SEQUENCE LISTING (9 sequences)

SEQ ID NO: 1 - protein, 307 aa, Artificial Sequence
  Ancestral protein of Renilla reniformis luciferase
MVSASQRTTSTATGDEWWAKCKQVDVLDSEMSYYDSDPGKHKNTVIFLHGNPTSSYLWRNVIPHVEPLARCLAPDLIGMGKSGKLPNHSYRFVDHYRYLSAWFDSVNLPEKVTIVCHDWGSGLGFHWCNEHRDRVKGIVHMESVVSPLKGWESFPETARDIFQALRSEAGEEMVLKKNFFIERLLPSSIMRKLSEEEMDAYREPFVEPGESRRPTLTWPREIPIKGDGPEDVIEIVKSYNKWLSTSKDIPKLFINADPGFFSNAIKKVTKNWPNQKTVTVKGLHFLQEDSPEEIGEAIADFLNELTK

SEQ ID NO: 2 - DNA, 918 bp, Artificial Sequence
  Nucleic acid sequence encoding the amino acid sequence shown for SEQ ID NO: 6
atggttagcgcaagccagcgtaccaccagtaccgcaaccggtgatgaatggtgggcaaaatgtaaacaggttgatgttctggatagcgagatgagctattatgatagcgatccgggtaaacataaaaacaccgtgatttttctgcatggtaatccgaccagcagctatctgtggcgtaatgttattccgcatgttgaaccgctggcacgttgtctggcaccggatctgattggtatgggtaaaagcggtaaactgccgaatcatagctatcgttttgtggatcattatcgttatctgagcgcatggtttgatagcgttaatctgccggaaaaagttaccattgtttgtcatgattggggtagcggtctgggttttcattggtgtaatgaacatcgtgatcgcgtgaaaggtattgttcacatggaaagcgttgtggatgttattgaaagctgggatgaatggcctgatatcgaagaagatattgccctgattaaaagcgaagccggtgaagaaatggttctgaaaaaaaactttttcatcgaacgtctgctgccgagcagcattatgcgtaaactgagcgaagaagagatggacgcatatcgtgaaccgtttgtggaaccgggtgaaagccgtcgtccgaccctgacctggcctcgtgaaattccgattaaaggtgatggtccggaagatgtgattgaaattgtgaaaagctacaacaaatggctgagcaccagcaaagatattccgaaactgtttattaacgcagaccctggcttttttagcaacgccatcaaaaaagtgaccaaaaattggccgaatcagaaaaccgttaccgttaaaggtctgcactttctgcaagaagattcaccggaagaaattggtgaagcaattgccgattttctgaacgaactgaccaaa

SEQ ID NO: 3 - DNA, 918 bp, Artificial Sequence; identical to SEQ ID NO: 2
  Nucleic acid sequence encoding the amino acid sequence shown for SEQ ID NO:7

SEQ ID NO: 4 - DNA, 918 bp, Artificial Sequence
  Nucleic acid sequence encoding the amino acid sequence shown for SEQ ID NO:8
atggttagcgcaagccagcgtaccaccagtaccgcaaccggtgatgaatggtgggcaaaatgtaaacaggttgatgttctggatagcgagatgagctattatgatagcgatccgggtaaacataaaaacaccgtgatttttctgcatggtaatccgaccagcagctatctgtggcgtaatgttattccgcatgttgaaccgctggcacgttgtctggcaccggatctgattggtatgggtaaaagcggtaaactgccgaatcatagctatcgttttgtggatcattatcgttatctgagcgcatggtttgatagcgttaatctgccggaaaaagttaccattgtttgtcatgattggggtagcggtctgggttttcattggtgtaatgaacatcgtgatcgcgtgaaaggtattgttcacatggaaagcgttgtggatgttattgaaagctgggatgaatggcctgatatcgaagaagccattgccctgattaaaagcgaagccggtgaagaaatggttctgaaaaaaaactttttcatcgaacgtctgctgccgagcagcattatgcgtaaactgagcgaagaagagatggacgcatatcgtgaaccgtttgtggaaccgggtgaaagccgtcgtccgaccctgacctggcctcgtgaaattccgattaaaggtgatggtccggaagatgtgattgaaattgtgaaaagctacaacaaatggctgagcaccagcaaagatattccgaaactgtttattaacgcagaccctggcttttttagcaacgccatcaaaaaagtgaccaaaaattggccgaatcagaaaaccgttaccgttaaaggtctgcactttctgcaagaagattcaccggaagaaattggtgaagcaattgccgattttctgaacgaactgaccaaa

SEQ ID NO: 5 - DNA, 918 bp, Artificial Sequence
  Nucleic acid sequence encoding the amino acid sequence shown for SEQ ID NO:9
atggttagcgcaagccagcgtaccaccagtaccgcaaccggtgatgaatggtgggcaaaatgtaaacaggttgatgttctggatagcgagatgagctattatgatagcgatccgggtaaacataaaaacaccgtgatttttctgcatggtaatccgaccagcagctatctgtggcgtaatgttattccgcatgttgaaccgctggcacgttgtctggcaccggatctgattggtatgggtaaaagcggtaaactgccgaatcatagctatcgttttgtggatcattatcgttatctgagcgcatggtttgatagcgttaatctgccggaaaaagttaccattgtttgtcatgattggggtagcggtctgggttttcattggtgtaatgaacatcgtgatcgcgtgaaaggtattgttcacatggaaagcgttgtggatgttattgaaagctgggatgaatggcctgatatcgaagaagccattgccctgattaaaagcgaagccggtgaagaaatggttctgaaaaaaaactttttcatcgaacgtctgctgccgagcagcattatgcgtaaactgagcgaagaagagatggacgcatatcgtgaaccgtttgtggaaccgggtgaaagccgtcgtccgaccctgacctggcctcgtgaaattccgctggttaaaggtggtaaaccggatgtgattgaaattgtgaaaagctacaacaaatggctgagcaccagcaaagatattccgaaactgtttattaacgcagaccctggcttttttagcaacgccatcaaaaaagtgaccaaaaattggccgaatcagaaaaccgttaccgttaaaggtctgcactttctgcaagaagattcaccggaagaaattggtgaagcaattgccgattttctgaacgaactgaccaaa

SEQ ID NO: 6 - protein, 306 aa, Artificial Sequence
  Amino acid sequence of AncFT
MVSASQRTTSTATGDEWWAKCKQVDVLDSEMSYYDSDPGKHKNTVIFLHGNPTSSYLWRNVIPHVEPLARCLAPDLIGMGKSGKLPNHSYRFVDHYRYLSAWFDSVNLPEKVTIVCHDWGSGLGFHWCNEHRDRVKGIVHMESVVDVIESWDEWPDIEEDIALIKSEAGEEMVLKKNFFIERLLPSSIMRKLSEEEMDAYREPFVEPGESRRPTLTWPREIPIKGDGPEDVIEIVKSYNKWLSTSKDIPKLFINADPGFFSNAIKKVTKNWPNQKTVTVKGLHFLQEDSPEEIGEAIADFLNELTK

SEQ ID NO: 7 - protein, 306 aa, Artificial Sequence
  Amino acid sequence of AncFT-L14
MVSASQRTTSTATGDEWWAKCKQVDVLDSEMSYYDSDPGKHKNTVIFLHGNPTSSYLWRNVIPHVEPLARCLAPDLIGMGKSGKLPNHSYRFVDHYRYLSAWFDSVNLPEKVTIVCHDWGSGLGFHWCNEHRDRVKGIVHMESVVDVIESWDEWPDIEEDIALIKSEAGEEMVLKKNFFIERLLPSSIMRKLSEEEMDAYREPFVEPGESRRPTLTWPREIPLVKGGKPDVIEIVKSYNKWLSTSKDIPKLFINADPGFFSNAIKKVTKNWPNQKTVTVKGLHFLQEDSPEEIGEAIADFLNELTK

SEQ ID NO: 8 - protein, 306 aa, Artificial Sequence
  Amino acid sequence of AncFT-D160A
MVSASQRTTSTATGDEWWAKCKQVDVLDSEMSYYDSDPGKHKNTVIFLHGNPTSSYLWRNVIPHVEPLARCLAPDLIGMGKSGKLPNHSYRFVDHYRYLSAWFDSVNLPEKVTIVCHDWGSGLGFHWCNEHRDRVKGIVHMESVVDVIESWDEWPDIEEAIALIKSEAGEEMVLKKNFFIERLLPSSIMRKLSEEEMDAYREPFVEPGESRRPTLTWPREIPIKGDGPEDVIEIVKSYNKWLSTSKDIPKLFINADPGFFSNAIKKVTKNWPNQKTVTVKGLHFLQEDSPEEIGEAIADFLNELTK

SEQ ID NO: 9 - protein, 306 aa, Artificial Sequence
  AncFT-L14-D160A
MVSASQRTTSTATGDEWWAKCKQVDVLDSEMSYYDSDPGKHKNTVIFLHGNPTSSYLWRNVIPHVEPLARCLAPDLIGMGKSGKLPNHSYRFVDHYRYLSAWFDSVNLPEKVTIVCHDWGSGLGFHWCNEHRDRVKGIVHMESVVDVIESWDEWPDIEEAIALIKSEAGEEMVLKKNFFIERLLPSSIMRKLSEEEMDAYREPFVEPGESRRPTLTWPREIPLVKGGKPDVIEIVKSYNKWLSTSKDIPKLFINADPGFFSNAIKKVTKNWPNQKTVTVKGLHFLQEDSPEEIGEAIADFLNELTK